European Patent Application EP 4 722 233 A1, published April 8, 2026. Title: METHOD TO IMPROVE PLANT GERMINATION AND FRUIT QUALITY UNDER STRESS CONDITIONS. Applicant: Universidad Politecnica de Madrid. The sequence listing filed with the application follows.

SEQUENCE LISTING (3 sequences)

SEQ ID NO: 1 - DNA, 934 bp, Arabidopsis sp.
  source 1..934: mol_type = genomic DNA
tacaattacattattcacgctgttttgtatactatgtaatttatataatgtcaaaaaagacggattataatgcccatattacccttctaacaaaaaataaaataaaataataatatccatattaccctttgacaatttcgagtataccatatgaattataacttagtattaaaatattgatttactccaacgacatattttaaaaatcaaatgatatatggtcaattatttagttttgaaagtgaattaatattagaagccaaaaacctagggccgccattagggttggtttgcctgttttgttgttatccaatatccaattcttattgtgcattgattccaatacaaatacaacactgagagtaattagaaaatggcatatttcttatatatatgtctgcgtgataaataaatggagtggttaagcattagtcatgttcttccaaatattacacctcaccgcatatgcagtagttttggcattacactaattcattaataacaaaagaaattatccttatgtaaattatgacgcaaatctttttattttattaatcggtacacgaaaaaaatcttttaataattcatgcatgtgataaaaacattgttaataatttaattttgattataatgataattgttttggataactatacatacatacgaagaagtcgtaaaacctttgaaagattttgcgatgacgatttaatgtcacgtgtctgcttgtgattgggtactttacgtgtgtaaaaagtaaggagcgcgccaacacaaaataacccattaagcttacgtgtcaagaagtgattggagaggacactctaccgaggctaaatacgaatcatactgaagcacatataaatagacgacgaacttcatactcttccaaataaactaacaaacgagatcgaagaagagttctcaacaacgaaaa

SEQ ID NO: 2 - DNA, 1674 bp, Arabidopsis sp.
  source 1..1674: mol_type = genomic DNA
atggcggaagaagcaaaatccaaaggaaacgcagctttctcttccggcgattacgccaccgcaataacccatttcacagaagcaatcaacctttcaccaaccaatcacatcctctactcaaacagatccgcttcttacgcttctctccaccgttacgaagaagctttatcagacgcgaagaagactatagagcttaaacctgattggtctaaaggatatagccgattaggtgctgcgtttattggattgtccaagtttgatgaagcggttgattcgtataagaaaggattagagattgatccgagtaatgagatgcttaaatcgggattagctgatgcttcgagatctagggtttcgtcaaagtcgaatccttttgttgatgcgtttcaagggaaggagatgtgggagaagttgacggcggatccggggactagggtttatttggagcaggatgattttgttaagacgatgaaggagattcagaggaaccctaataatcttaatttgtatatgaaggataagagagttatgaaggctttaggggttttgttgaatgtgaagtttggtggatctagtggtgaagatactgagatgaaggaggctgatgagaggaaagagcctgaaccggagatggaacctatggagttgacggaggaggagaggcagaagaaggagagaaaggagaaggctttgaaggagaaaggggaaggaaatgttgcttataagaagaaggattttgggagagctgttgaacattatactaaggccatggagctcgatgatgaggatatttcgtatttgacgaatcgtgctgctgtttatcttgagatggggaagtacgaggagtgcattgaagactgtgacaaggctgttgaaagaggcagagaacttcgttctgacttcaagatgatagcaagagctctgactagaaaaggatctgctctagtgaaaatggcgagatgctcgaaagactttgagcctgcgattgagactttccagaaagctcttacagagcatcgtaatccagatacattgaagaaactgaacgatgctgagaaagtcaagaaagagctggagcaacaggagtactttgatcctacgatagccgaggaggagcgagagaaaggtaatggattctttaaagaacaaaagtatccagaggcagtgaagcattattcagaagcaatcaaaagaaacccgaacgacgtgagggcatatagcaacagagctgcttgttacacaaagttaggagcattaccagagggattgaaagatgctgaaaaatgcattgagctggacccaagtttcacgaaaggatacagtagaaaaggagctattcaatttttcatgaaggaatacgataaagctatggaaacgtatcaagaagggctaaaacatgatcctaagaaccaggagttccttgatggtgttagaagatgtgtggaacagataaacaaagcgagccgtggtgatctgactccagaagaattgaaggagagacaagcaaaggcaatgcaagatcctgaagttcagaacatattatcggatccagtgatgagacaggtactagtggactttcaagagaatccgaaagctgcacaagagcatatgaagaacccaatggtaatgaacaagattcagaagctggttagtgccggaattgttcaggtccgg

SEQ ID NO: 3 - DNA, 2785 bp, synthetic construct
  source 1..2785: mol_type = other DNA
tacaattacattattcacgctgttttgtatactatgtaatttatataatgtcaaaaaagacggattataatgcccatattacccttctaacaaaaaataaaataaaataataatatccatattaccctttgacaatttcgagtataccatatgaattataacttagtattaaaatattgatttactccaacgacatattttaaaaatcaaatgatatatggtcaattatttagttttgaaagtgaattaatattagaagccaaaaacctagggccgccattagggttggtttgcctgttttgttgttatccaatatccaattcttattgtgcattgattccaatacaaatacaacactgagagtaattagaaaatggcatatttcttatatatatgtctgcgtgataaataaatggagtggttaagcattagtcatgttcttccaaatattacacctcaccgcatatgcagtagttttggcattacactaattcattaataacaaaagaaattatccttatgtaaattatgacgcaaatctttttattttattaatcggtacacgaaaaaaatcttttaataattcatgcatgtgataaaaacattgttaataatttaattttgattataatgataattgttttggataactatacatacatacgaagaagtcgtaaaacctttgaaagattttgcgatgacgatttaatgtcacgtgtctgcttgtgattgggtactttacgtgtgtaaaaagtaaggagcgcgccaacacaaaataacccattaagcttacgtgtcaagaagtgattggagaggacactctaccgaggctaaatacgaatcatactgaagcacatataaatagacgacgaacttcatactcttccaaataaactaacaaacgagatcgaagaagagttctcaacaacgaaaaacaactttgtatacaaaagttgtccccatggcggaagaagcaaaatccaaaggaaacgcagctttctcttccggcgattacgccaccgcaataacccatttcacagaagcaatcaacctttcaccaaccaatcacatcctctactcaaacagatccgcttcttacgcttctctccaccgttacgaagaagctttatcagacgcgaagaagactatagagcttaaacctgattggtctaaaggatatagccgattaggtgctgcgtttattggattgtccaagtttgatgaagcggttgattcgtataagaaaggattagagattgatccgagtaatgagatgcttaaatcgggattagctgatgcttcgagatctagggtttcgtcaaagtcgaatccttttgttgatgcgtttcaagggaaggagatgtgggagaagttgacggcggatccggggactagggtttatttggagcaggatgattttgttaagacgatgaaggagattcagaggaaccctaataatcttaatttgtatatgaaggataagagagttatgaaggctttaggggttttgttgaatgtgaagtttggtggatctagtggtgaagatactgagatgaaggaggctgatgagaggaaagagcctgaaccggagatggaacctatggagttgacggaggaggagaggcagaagaaggagagaaaggagaaggctttgaaggagaaaggggaaggaaatgttgcttataagaagaaggattttgggagagctgttgaacattatactaaggccatggagctcgatgatgaggatatttcgtatttgacgaatcgtgctgctgtttatcttgagatggggaagtacgaggagtgcattgaagactgtgacaaggctgttgaaagaggcagagaacttcgttctgacttcaagatgatagcaagagctctgactagaaaaggatctgctctagtgaaaatggcgagatgctcgaaagactttgagcctgcgattgagactttccagaaagctcttacagagcatcgtaatccagatacattgaagaaactgaacgatgctgagaaagtcaagaaagagctggagcaacaggagtactttgatcctacgatagccgaggaggagcgagagaaaggtaatggattctttaaagaacaaaagtatccagaggcagtgaagcattattcagaagcaatcaaaagaaacccgaacgacgtgagggcatatagcaacagagctgcttgttacacaaagttaggagcattaccagagggattgaaagatgctgaaaaatgcattgagctggacccaagtttcacgaaaggatacagtagaaaaggagctattcaatttttcatgaaggaatacgataaagctatggaaacgtatcaagaagggctaaaacatgatcctaagaaccaggagttccttgatggtgttagaagatgtgtggaacagataaacaaagcgagccgtggtgatctgactccagaagaattgaaggagagacaagcaaaggcaatgcaagatcctgaagttcagaacatattatcggatccagtgatgagacaggtactagtggactttcaagagaatccgaaagctgcacaagagcatatgaagaacccaatggtaatgaacaagattcagaagctggttagtgccggaattgttcaggtccggtacccagctttcttgtacaaagtggtccccgggttaattaacatcttttacccatacgatgttcctgactatgcgggctatccctatgacgtcccggactatgcaggatcctatccatatgacgttccagattacgctgctcagtgcagc